European Patent Specification EP 3 974 830 B1, published September 10, 2025. Title: POLYPEPTIDE MAGNETIC NANOPARTICLE, PREPARATION METHOD THEREFOR AND USE THEREOF. Applicant: BEIJING NANOPEP BIOTECH CORPORATION, LTD. The sequence listing filed with the application follows.

SEQUENCE LISTING (9 sequences)

SEQ ID NO: 1 - protein, 26 aa, Artificial Sequence
VRRDAPRFSMQGLDACGGNNCNNNNN

SEQ ID NO: 4 - protein, 25 aa, Artificial Sequence
VRRDAPRFSMQGLDACGGNNCNNNN

SEQ ID NO: 3 - protein, 24 aa, Artificial Sequence
VRRDAPRFSMQGLDACGGNNCNNN

SEQ ID NO: 4 - protein, 25 aa, Artificial Sequence
VRRDAPRFSMQGLDACGGCNNNNNN

SEQ ID NO: 5 - protein, 24 aa, Artificial Sequence
VRRDAPRFSMQGLDACGGCNNNNN

SEQ ID NO: 6 - protein, 23 aa, Artificial Sequence
VRRDAPRFSMQGLDACGGCNNNN

SEQ ID NO: 7 - protein, 25 aa, Artificial Sequence
VRRDAPRFSMQGLDAGGCNNCNNNN

SEQ ID NO: 8 - protein, 24 aa, Artificial Sequence
VRRDAPRFSMQGLDAGGCNNCNNN

SEQ ID NO: 9 - protein, 23 aa, Artificial Sequence
VRRDAPRFSMQGLDAGGCNNCNN